European Patent Specification EP 3 530 284 B1, published October 25, 2023. Title: ANTI-INTEGRIN B1 ANTIBODY COMPOSITIONS AND METHODS OF USE THEREOF. Applicant: ONCOSYNERGY, INC. CARBONELL, W. Shawn. The sequence listing filed with the application follows.

SEQUENCE LISTING (125 sequences)

SEQ ID NO: 1 - DNA, 363 bp, Artificial Sequence
  Synthetic construct
gaagtccagctgcagcagtctgggcctgaggttgggaggcctgggtcctcagtcaagatttcttgcaaggcttctggctacacctttaccgggtacattttgagctgggtgaagcagagtcctggacaggggctggaatggataggatgggttgatcctgaatatggtagtactgattctgctgagaagttcaaaaagagggccacactgactgcagatatatcctccaacacagcctacatccagcttagcagcctgacatctgaggacacagccacctatttttgtactagatattatgatggttattatcgccggtggtttgcttactggggccaaggcactctggtcactgtctcttca

SEQ ID NO: 2 - protein, 121 aa, Artificial Sequence
  Synthetic construct
EVQLQQSGPEVGRPGSSVKISCKASGYTFTGYILSWVKQSPGQGLEWIGWVDPEYGSTDSAEKFKKRATLTADISSNTAYIQLSSLTSEDTATYFCTRYYDGYYRRWFAYWGQGTLVTVSS

SEQ ID NO: 3 - DNA, 321 bp, Artificial Sequence
  Synthetic construct
gacatccagatgacacagtctccagcttccctgtctgcatctctgggagacattgtctccatcgaatgtcttgcaagtgagggcatttccaataatttagcgtggcatcagcagaagccagggaaatctcctcagctcctgatctatggtgcacatagcttacatgacggggtcccatcacggttcagtggcagtggatctggcacacagtattctctcaagatcagcggcatgcaacctgaagatgaaggggtttattactgtcaacagggttacaaatatccgatcacgtttggaggtgggaccaagctggaactgaaa

SEQ ID NO: 4 - protein, 107 aa, Artificial Sequence
  Synthetic construct
DIQMTQSPASLSASLGDIVSIECLASEGISNNLAWHQQKPGKSPQLLIYGAHSLHDGVPSRFSGSGSGTQYSLKISGMQPEDEGVYYCQQGYKYPITFGGGTKLELK

SEQ ID NO: 5 - DNA, 363 bp, Artificial Sequence
  Synthetic construct
gaggtgcagctggtgcagtccggccccgaggtgaagaagcccggctcctccgtgaagatctcctgcaaggcctccggctacaccttcaccggctacatcctgtcctgggtgaagcaggcccccggccagggcctggagtggatcggctgggtggaccccgagtacggctccaccgactccgccgagaagttcaagaagcgcgccaccctgaccgccgacatctccaccaacaccgcctacatccagctgtcctccctgcgctccgaggacaccgccacctacttctgcacccgctactacgacggctactaccgccgctggttcgcctactggggccagggcaccctggtgaccgtgtcctcc

SEQ ID NO: 6 - protein, 121 aa, Artificial Sequence
  Synthetic construct
EVQLVQSGPEVKKPGSSVKISCKASGYTFTGYILSWVKQAPGQGLEWIGWVDPEYGSTDSAEKFKKRATLTADISTNTAYIQLSSLRSEDTATYFCTRYYDGYYRRWFAYWGQGTLVTVSS

SEQ ID NO: 7 - DNA, 363 bp, Artificial Sequence
  Synthetic construct
gaggtgcagctggtgcagtccggcgccgaggtgaagaagcccggctcctccgtgaagatctcctgcaaggcctccggctacaccttcaccggctacatcctgtcctgggtgcgccaggcccccggccagggcctggagtggatcggctgggtggaccccgagtacggctccaccgactccgccgagaagttcaagaagcgcgccaccctgaccgccgacatctccaccaacaccgcctacatcgagctgtcctccctgcgctccgaggacaccgccacctacttctgcacccgctactacgacggctactaccgccgctggttcgcctactggggccagggcaccctggtgaccgtgtcctcc

SEQ ID NO: 8 - protein, 121 aa, Artificial Sequence
  Synthetic construct
EVQLVQSGAEVKKPGSSVKISCKASGYTFTGYILSWVRQAPGQGLEWIGWVDPEYGSTDSAEKFKKRATLTADISTNTAYIELSSLRSEDTATYFCTRYYDGYYRRWFAYWGQGTLVTVSS

SEQ ID NO: 9 - DNA, 363 bp, Artificial Sequence
  Synthetic construct
gaggtgcagctggtgcagtccggcgccgaggtgaagaagcccggctcctccgtgaagatctcctgcaaggcctccggctacaccttcaccggctacatcctgtcctgggtgcgccaggcccccggccagggcctggagtggatcggctgggtggaccccgagtacggctccaccgactccgccgagaagttcaagaagcgcgccaccctgaccgccgacatctccacctccaccgcctacatcgagctgtcctccctgcgctccgaggacaccgccacctacttctgcacccgctactacgacggctactaccgccgctggttcgcctactggggccagggcaccctggtgaccgtgtcctcc

SEQ ID NO: 10 - protein, 121 aa, Artificial Sequence
  Synthetic construct
EVQLVQSGAEVKKPGSSVKISCKASGYTFTGYILSWVRQAPGQGLEWIGWVDPEYGSTDSAEKFKKRATLTADISTSTAYIELSSLRSEDTATYFCTRYYDGYYRRWFAYWGQGTLVTVSS

SEQ ID NO: 11 - DNA, 363 bp, Artificial Sequence
  Synthetic construct
gaggtgcagctggtgcagtccggcgccgaggtgaagaagcccggctcctccgtgaaggtgtcctgcaaggcctccggctacaccttcaccggctacatcctgtcctgggtgcgccaggcccccggccagggcctggagtggatcggctgggtggaccccgagtacggctccaccgactccgccgagaagttcaagaagcgcgccaccatcaccgccgacatctccacctccaccgcctacatggagctgtcctccctgcgctccgaggacaccgccacctacttctgcacccgctactacgacggctactaccgccgctggttcgcctactggggccagggcaccctggtgaccgtgtcctcc

SEQ ID NO: 12 - protein, 121 aa, Artificial Sequence
  Synthetic construct
EVQLVQSGAEVKKPGSSVKVSCKASGYTFTGYILSWVRQAPGQGLEWIGWVDPEYGSTDSAEKFKKRATITADISTSTAYMELSSLRSEDTATYFCTRYYDGYYRRWFAYWGQGTLVTVSS

SEQ ID NO: 13 - DNA, 363 bp, Artificial Sequence
  Synthetic construct
gaggtgcagctggtgcagtccggcgccgaggtgaagaagcccggctcctccgtgaaggtgtcctgcaaggcctccggctacaccttcaccggctacatcctgtcctgggtgcgccaggcccccggccagggcctggagtggatcggctgggtggaccccgagtacggctccaccgactccgccgagaagttcaagaagcgcgtgaccatcaccgccgacatctccacctccaccgcctacatggagctgtcctccctgcgctccgaggacaccgccacctacttctgcacccgctactacgacggctactaccgccgctggttcgcctactggggccagggcaccctggtgaccgtgtcctcc

SEQ ID NO: 14 - protein, 121 aa, Artificial Sequence
  Synthetic construct
EVQLVQSGAEVKKPGSSVKVSCKASGYTFTGYILSWVRQAPGQGLEWIGWVDPEYGSTDSAEKFKKRVTITADISTSTAYMELSSLRSEDTATYFCTRYYDGYYRRWFAYWGQGTLVTVSS

SEQ ID NO: 15 - DNA, 321 bp, Artificial Sequence
  Synthetic construct
gacatccagatgacccagtccccctcctccctgtccgcctccgtgggcgaccgcgtgaccatcacctgcctggcctccgagggcatctccaacaacctggcctggcaccagcagaagcccggcaaggccccccagctgctgatctacggcgcccactccctgcacgacggcgtgcccgaccgcttctccggctccggctccggcaccgactacaccctgaagatctccggcatgcagcccgaggacgagggcgtgtactactgccagcagggctacaagtaccccatcaccttcggcggcggcaccaaggtggagatcaag

SEQ ID NO: 16 - protein, 107 aa, Artificial Sequence
  Synthetic construct
DIQMTQSPSSLSASVGDRVTITCLASEGISNNLAWHQQKPGKAPQLLIYGAHSLHDGVPDRFSGSGSGTDYTLKISGMQPEDEGVYYCQQGYKYPITFGGGTKVEIK

SEQ ID NO: 17 - DNA, 321 bp, Artificial Sequence
  Synthetic construct
gacatccagatgacccagtccccctcctccctgtccgcctccgtgggcgaccgcgtgaccatcacctgcctggcctccgagggcatctccaacaacctggcctggcaccagcagaagcccggcaaggcccccaagctgctgatctacggcgcccactccctgcacgacggcgtgcccgaccgcttctccggctccggctccggcaccgactacaccctgaagatctcccgcgtggaggccgaggacgtgggcgtgtactactgccagcagggctacaagtaccccatcaccttcggcggcggcaccaaggtggagatcaag

SEQ ID NO: 18 - protein, 107 aa, Artificial Sequence
  Synthetic construct
DIQMTQSPSSLSASVGDRVTITCLASEGISNNLAWHQQKPGKAPKLLIYGAHSLHDGVPDRFSGSGSGTDYTLKISRVEAEDVGVYYCQQGYKYPITFGGGTKVEIK

SEQ ID NO: 19 - DNA, 321 bp, Artificial Sequence
  Synthetic construct
gacatccagatgacccagtccccctcctccctgtccgcctccgtgggcgaccgcgtgaccatcacctgcctggcctccgagggcatctccaacaacctggcctggtaccagcagaagcccggcaaggcccccaagctgctgatctacggcgcccactccctgcacgacggcgtgcccgaccgcttctccggctccggctccggcaccgactacaccctgaagatctcccgcgtggaggccgaggacgtgggcgtgtactactgccagcagggctacaagtaccccatcaccttcggcggcggcaccaaggtggagatcaag

SEQ ID NO: 20 - protein, 107 aa, Artificial Sequence
  Synthetic construct
DIQMTQSPSSLSASVGDRVTITCLASEGISNNLAWYQQKPGKAPKLLIYGAHSLHDGVPDRFSGSGSGTDYTLKISRVEAEDVGVYYCQQGYKYPITFGGGTKVEIK

SEQ ID NO: 21 - DNA, 321 bp, Artificial Sequence
  Synthetic construct
gacatccagatgacccagtccccctcctccctgtccgcctccgtgggcgaccgcgtgaccatcacctgcctggcctccgagggcatctccaacaacctggcctggtaccagcagaagcccggcaaggcccccaagctgctgatctacggcgcccactccctgcacgacggcgtgcccgaccgcttctccggctccggctccggcaccgacttcaccctgaagatctcccgcgtggaggccgaggacgtgggcgtgtactactgccagcagggctacaagtaccccatcaccttcggcggcggcaccaaggtggagatcaag

SEQ ID NO: 22 - protein, 107 aa, Artificial Sequence
  Synthetic construct
DIQMTQSPSSLSASVGDRVTITCLASEGISNNLAWYQQKPGKAPKLLIYGAHSLHDGVPDRFSGSGSGTDFTLKISRVEAEDVGVYYCQQGYKYPITFGGGTKVEIK

SEQ ID NO: 23 - protein, 5 aa, Artificial Sequence
  Synthetic construct
GYILS

SEQ ID NO: 24 - protein, 17 aa, Artificial Sequence
  Synthetic construct
WVDPEYGSTDSAEKFKK

SEQ ID NO: 25 - protein, 12 aa, Artificial Sequence
  Synthetic construct
YYDGYYRRWFAY

SEQ ID NO: 26 - protein, 11 aa, Artificial Sequence
  Synthetic construct
LASEGISNNLA

SEQ ID NO: 27 - protein, 7 aa, Artificial Sequence
  Synthetic construct
GAHSLHD

SEQ ID NO: 28 - protein, 9 aa, Artificial Sequence
  Synthetic construct
QQGYKYPIT

SEQ ID NO: 29 - protein, 121 aa, Artificial Sequence
  Synthetic construct
EVQLVQSGPEVKKPGASVKISCKASGYTFTGYILSWVKQAPGKGLEWIGWVDPEYGSTDSAEKFKKRATLTADISANTAYIQLSSLTSEDTATYFCTRYYDGYYRRWFAYWGQGTLVTVSS

SEQ ID NO: 30 - protein, 121 aa, Artificial Sequence
  Synthetic construct
EVQLVQSGAEVKKPGASVKISCKASGYTFTGYILSWVRQAPGKGLEWIGWVDPEYGSTDSAEKFKKRATLTADISANTAYIELSSLTSEDTATYFCTRYYDGYYRRWFAYWGQGTLVTVSS

SEQ ID NO: 31 - protein, 121 aa, Artificial Sequence
  Synthetic construct
EVQLVQSGAEVKKPGASVKISCKASGYTFTGYILSWVRQAPGKGLEWIGWVDPEYGSTDSAEKFKKRATLTADISASTAYIELSSLTSEDTATYFCTRYYDGYYRRWFAYWGQGTLVTVSS

SEQ ID NO: 32 - protein, 121 aa, Artificial Sequence
  Synthetic construct
EVQLVQSGAEVKKPGASVKVSCKASGYTFTGYILSWVRQAPGKGLEWIGWVDPEYGSTDSAEKFKKRATITADISASTAYMELSSLTSEDTATYFCTRYYDGYYRRWFAYWGQGTLVTVSS

SEQ ID NO: 33 - protein, 121 aa, Artificial Sequence
  Synthetic construct
EVQLVQSGAEVKKPGASVKVSCKASGYTFTGYILSWVRQAPGKGLEWIGWVDPEYGSTDSAEKFKKRVTITADISASTAYMELSSLTSEDTATYFCTRYYDGYYRRWFAYWGQGTLVTVSS

SEQ ID NO: 34 - protein, 121 aa, Artificial Sequence
  Synthetic construct
EVQLVQSGPEVKKPGASVKISCKASGYTFTGYILSWVKQAPGKGLEWIGWVDPEYGSTDSAEKFKKRATLTADISKNTAYIQLNSLTAEDTATYFCTRYYDGYYRRWFAYWGQGTLVTVSS

SEQ ID NO: 35 - protein, 121 aa, Artificial Sequence
  Synthetic construct
EVQLVQSGAEVKKPGASVKISCKASGYTFTGYILSWVRQAPGKGLEWIGWVDPEYGSTDSAEKFKKRATLTADISKNTAYIQLNSLTAEDTATYFCTRYYDGYYRRWFAYWGQGTLVTVSS

SEQ ID NO: 36 - protein, 121 aa, Artificial Sequence
  Synthetic construct
EVQLVQSGAEVKKPGASVKVSCKASGYTFTGYILSWVRQAPGKGLEWIGWVDPEYGSTDSAEKFKKRATLTADISKNTAYIQLNSLTAEDTATYFCTRYYDGYYRRWFAYWGQGTLVTVSS

SEQ ID NO: 37 - protein, 121 aa, Artificial Sequence
  Synthetic construct
EVQLVQSGAEVKKPGASVKVSCKASGYTFTGYILSWVRQAPGKGLEWIGWVDPEYGSTDSAEKFKKRATITADISKNTAYLQLNSLTAEDTATYFCTRYYDGYYRRWFAYWGQGTLVTVSS

SEQ ID NO: 38 - protein, 121 aa, Artificial Sequence
  Synthetic construct
EVQLVQSGAEVKKPGASVKVSCKVSGYTFTGYILSWVRQAPGKGLEWIGWVDPEYGSTDSAEKFKKRFTITADISKNTAYLQMNSLTAEDTATYFCTRYYDGYYRRWFAYWGQGTLVTVSS

SEQ ID NO: 39 - protein, 97 aa, Artificial Sequence
  Synthetic construct
QVQLQESGPGLVKPSETLSLICAVSGDSISSGNWIWVRQPPGKGLEWIGEIHHSGSTYYNPSLKSRITMSVDTSKNQFYLKLSSVTAADTAVYYCAR

SEQ ID NO: 40 - protein, 97 aa, Artificial Sequence
  Synthetic construct
QVQLQQWGAGLLKPSETLSLTCAVYGGSFSGYYWSWIRQPPGKGLEWIGEINHSGSTNNNPSLKSRATISVDTSKNQFSLKLSSVTAADTAVYYCAR

SEQ ID NO: 41 - protein, 98 aa, Artificial Sequence
  Synthetic construct
EVQLVQSGAEVKKPGESLKISCKGSGYSFTSYWIGWVRQMPGKGLEWMGIIYPGDSDTRYSPSFQGQVTISADKSISTAYLQWSSLKASDTAMYYCAR

SEQ ID NO: 42 - protein, 98 aa, Artificial Sequence
  Synthetic construct
QVQLQQSGPGLVKPSQTLSLTCAISGDSSNSAAWNWIRQSPSRGLEWLGRTYYSKWYNDYAVSVKSRITINPDTSKNQFSLQLNSVTPEDTAVYYCAR

SEQ ID NO: 43 - protein, 98 aa, Artificial Sequence
  Synthetic construct
QVQLVQSGSELKKPGASVKVSCKASGYTFTSYAMNWVRQAPGQGLEWMGWINTNTGNPTYAQGFTGRFVFSLDTSVSTAYLQICSLKAEDTAVYYCAR

SEQ ID NO: 44 - protein, 107 aa, Artificial Sequence
  Synthetic construct
DIQMTQSPDSLSASLGDRATINCLASEGISNNLAWHQQKPGQSPQLLIYGAHSLHDGVPSRFSGSGSGTEYTLKISGMQPEDEAVYYCQQGYKYPITFGGGTKVEIK

SEQ ID NO: 45 - protein, 107 aa, Artificial Sequence
  Synthetic construct
DIQMTQSPDSLSASLGDRATINCLASEGISNNLAWHQQKPGQSPRLLIYGAHSLHDGVPSRFSGSGSGTEYTLKISSMQPEDFAVYYCQQGYKYPITFGGGTKVEIK

SEQ ID NO: 46 - protein, 107 aa, Artificial Sequence
  Synthetic construct
DIVMTQSPDSLSASLGDRATINCLASEGISNNLAWHQQKPGQSPRLLIYGAHSLHDGVPSRFSGSGSGTEYTLKISSMQPEDFAVYYCQQGYKYPITFGGGTKVEIK

SEQ ID NO: 47 - protein, 107 aa, Artificial Sequence
  Synthetic construct
DIVMTQSPDSLSASLGDRATINCLASEGISNNLAWYQQKPGQSPRLLIYGAHSLHDGVPSRFSGSGSGTEYTLKISSMQPEDFAVYYCQQGYKYPITFGGGTKVEIK

SEQ ID NO: 48 - protein, 107 aa, Artificial Sequence
  Synthetic construct
DIQMTQSPASLSASLGDIVSIECLASEGISNNLAWHQQKPGQSPQLLIYGAHSLHDGVPSRFSGSGSGTDYTLKISGMQPEDEGVYYCQQGYKYPITFGGGTKVEIK

SEQ ID NO: 49 - protein, 107 aa, Artificial Sequence
  Synthetic construct
DIQMTQSPASLSASLGDIVSIECLASEGISNNLAWHQQKPGQSPRLLIYGAHSLHDGVPSRFSGSGSGTDYTLKISRVEPEDVGVYYCQQGYKYPITFGGGTKVEIK

SEQ ID NO: 50 - protein, 107 aa, Artificial Sequence
  Synthetic construct
DIQMTQSPATLSASLGDIVSIECLASEGISNNLAWHQQKPGQSPRLLIYGAHSLHDGVPSRFSGSGSGTDYTLKISRVEAEDVGVYYCQQGYKYPITFGGGTKVEIK

SEQ ID NO: 51 - protein, 107 aa, Artificial Sequence
  Synthetic construct
EIQMTQSPATLSASLGDIVSIECLASEGISNNLAWHQQKPGQSPRLLIYGAHSLHDGVPSRFSGSGSGTDYTLKISRVEAEDVGVYYCQQGYKYPITFGGGTKVEIK

SEQ ID NO: 52 - protein, 107 aa, Artificial Sequence
  Synthetic construct
EIVMTQSPATLSASLGDIVSIECLASEGISNNLAWYQQKPGQSPRLLIYGAHSLHDGVPSRFSGSGSGTDYTLKISRVEAEDVGVYYCQQGYKYPITFGGGTKVEIK

SEQ ID NO: 53 - protein, 95 aa, Artificial Sequence
  Synthetic construct
VIWMTQSPSLLSASTGDRVTISCRMSQGISSYLAWYQQKPGKAPELLIYAASTLQSGVPSRFSGSGSGTDFTLTISCLQSEDFATYYCQQYYSFP

SEQ ID NO: 54 - protein, 95 aa, Artificial Sequence
  Synthetic construct
DVVMTQSPLSLPVTLGQPASISCRSSQDGNTYLNWFQQRPGQSPRRLIYKVSNWDSGVPDRFSGSGSGTDFTLKISRVEAEDVGVYYCMQGTHWP

SEQ ID NO: 55 - protein, 95 aa, Artificial Sequence
  Synthetic construct
EIVLTQSPGTLSLSPGERATLSCRASQVSSSYLAWYQQKPGQAPRLLIYGASSRATGIPDRFSGSGSGTDFTLTISRLEPEDFAVYYCQQYGSSP

SEQ ID NO: 56 - protein, 95 aa, Artificial Sequence
  Synthetic construct
DIVMTQSPDSLAVSLGERATINCKSSQNNKNYLAWYQQKPGQPPKLLIYWASTRESGVPDRFSGSGSGTDFTLTISSLQAEDVAVYYCQQYYSTP

SEQ ID NO: 57 - protein, 95 aa, Artificial Sequence
  Synthetic construct
DVVMTQSPAFLSVTPGEKVTITCQASEGIGNYLYWYQQKPDQAPKLLIKYASQSISGVPSRFSGSGSGTDFTFTISSLEAEDAATYYCQQGNKHP

SEQ ID NO: 58 - DNA, 25 bp, Artificial Sequence
  Primer
atgrasttskggytmarctkgrttt

SEQ ID NO: 59 - DNA, 26 bp, Artificial Sequence
  Primer
atgraatgsasctgggtywtyctctt

SEQ ID NO: 60 - DNA, 29 bp, Artificial Sequence
  Primer
atggactccaggctcaatttagttttcct

SEQ ID NO: 61 - DNA, 26 bp, Artificial Sequence
  Primer
atggctgtcytrgbgctgytcytctg

SEQ ID NO: 62 - DNA, 29 bp, Artificial Sequence
  Primer
atggvttggstgtggamcttgcyattcct

SEQ ID NO: 63 - DNA, 26 bp, Artificial Sequence
  Primer
atgaaatgcagctggrtyatsttctt

SEQ ID NO: 64 - DNA, 26 bp, Artificial Sequence
  Primer
atggrcagrcttacwtyytcattcct

SEQ ID NO: 65 - DNA, 26 bp, Artificial Sequence
  Primer
atgatggtgttaagtcttctgtacct

SEQ ID NO: 66 - DNA, 26 bp, Artificial Sequence
  Primer
atgggatggagctrtatcatsytctt

SEQ ID NO: 67 - DNA, 23 bp, Artificial Sequence
  Primer
atgaagwtgtggbtraactggrt

SEQ ID NO: 68 - DNA, 25 bp, Artificial Sequence
  Primer
  misc_feature (15)..(15): n is Inosine
atggratggasckknrtctttmtct

SEQ ID NO: 69 - DNA, 25 bp, Artificial Sequence
  Primer
atgaacttygggytsagmttgrttt

SEQ ID NO: 70 - DNA, 25 bp, Artificial Sequence
  Primer
atgtacttgggactgagctgtgtat

SEQ ID NO: 71 - DNA, 23 bp, Artificial Sequence
  Primer
atgagagtgctgattcttttgtg

SEQ ID NO: 72 - DNA, 28 bp, Artificial Sequence
  Primer
atggattttgggctgattttttttattg

SEQ ID NO: 73 - DNA, 26 bp, Artificial Sequence
  Primer
  misc_feature (21)..(21): n is Inosine
ccagggrccarkggataracngrtgg

SEQ ID NO: 74 - DNA, 24 bp, Artificial Sequence
  Primer
atgragwcacakwcycaggtcttt

SEQ ID NO: 75 - DNA, 25 bp, Artificial Sequence
  Primer
atggagacagacacactcctgctat

SEQ ID NO: 76 - DNA, 29 bp, Artificial Sequence
  Primer
atggagwcagacacactsctgytatgggt

SEQ ID NO: 77 - DNA, 32 bp, Artificial Sequence
  Primer
  misc_feature (27)..(27): n is Inosine
atgaggrcccctgctcagwttyttggnwtctt

SEQ ID NO: 78 - DNA, 30 bp, Artificial Sequence
  Primer
tgggcwtcaagatgragtcacakwyycwgg

SEQ ID NO: 79 - DNA, 29 bp, Artificial Sequence
  Primer
atgagtgtgcycactcaggtcctggsgtt

SEQ ID NO: 80 - DNA, 31 bp, Artificial Sequence
  Primer
atgtggggaycgktttyammcttttcaattg

SEQ ID NO: 81 - DNA, 28 bp, Artificial Sequence
  Primer
atggaagccccagctcagcttctcttcc

SEQ ID NO: 82 - DNA, 26 bp, Artificial Sequence
  Primer
  misc_feature (6)..(6): n is Inosine
  misc_feature (12)..(12): n is Inosine
  misc_feature (18)..(18): n is Inosine
atgagnmmktcnmttcanttcytggg

SEQ ID NO: 83 - DNA, 26 bp, Artificial Sequence
  Primer
  misc_feature (12)..(12): n is Inosine
  misc_feature (24)..(24): n is Inosine
atgakgthcycngctcagytyctnrg

SEQ ID NO: 84 - DNA, 25 bp, Artificial Sequence
  Primer
atggtrtccwcasctcagttccttg

SEQ ID NO: 85 - DNA, 27 bp, Artificial Sequence
  Primer
atgtatatatgtttgttgtctatttct

SEQ ID NO: 86 - DNA, 29 bp, Artificial Sequence
  Primer
atgaagttgcctgttaggctgttggtgct

SEQ ID NO: 87 - DNA, 29 bp, Artificial Sequence
  Primer
atggatttwcargtgcagattwtcagctt

SEQ ID NO: 88 - DNA, 27 bp, Artificial Sequence
  Primer
atggtyctyatvtccttgctgttctgg

SEQ ID NO: 89 - DNA, 27 bp, Artificial Sequence
  Primer
atggtyctyatvttrctgctgctatgg

SEQ ID NO: 90 - DNA, 21 bp, Artificial Sequence
  Primer
actggatggtgggaagatgga

SEQ ID NO: 91 - protein, 120 aa, Artificial Sequence
  Synthetic construct
QVQLQESGPGLVKPSETLSLICAVSGDSISSGNWIWVRQPPGKGLEWIGEIHHSGSTYYNPSLKSRITMSVDTSKNQFYLKLSSVTAADTAVYYCARYYDGYYRRWFAYWGRGTLVTVSS

SEQ ID NO: 92 - protein, 121 aa, Artificial Sequence
  Synthetic construct
EVQLQQSGPGLGRPGSSVKISCKASGYTFTGYILSWVRQPPGKGLEWIGWVDPEYGSTDSAEKFKKRATMSADISKNQAYLKLSSVTAADTATYYCTRYYDGYYRRWFAYWGRGTLVTVSS

SEQ ID NO: 93 - protein, 120 aa, Artificial Sequence
  Synthetic construct
QVQLQQWGAGLLKPSETLSLTCAVYGGSFSGYYWSWIRQPPGKGLEWIGEINHSGSTNNNPSLKSRATISVDTSKNQFSLKLSSVTAADTAVYYCARYYDGYYRRWFAYWGQGTLVTVSS

SEQ ID NO: 94 - protein, 121 aa, Artificial Sequence
  Synthetic construct
EVQLQQWGAGLGRPGSSVKISCKASGYTFTGYILSWVRQPPGKGLEWIGWVDPEYGSTDSAEKFKKRATISADISKNQAYLKLSSVTAADTATYYCTRYYDGYYRRWFAYWGQGTLVTVSS

SEQ ID NO: 95 - protein, 121 aa, Artificial Sequence
  Synthetic construct
EVQLVQSGAEVKKPGESLKISCKGSGYSFTSYWIGWVRQMPGKGLEWMGIIYPGDSDTRYSPSFQGQVTISADKSISTAYLQWSSLKASDTAMYYCARYYDGYYRRWFAYWGQGTLVTVSS

SEQ ID NO: 96 - protein, 121 aa, Artificial Sequence
  Synthetic construct
EVQLVQSGAEVGRPGSSVKISCKASGYTFTGYILSWVRQMPGKGLEWIGWVDPEYGSTDSAEKFKKRATLSADISINTAYLQLSSLKASDTATYYCTRYYDGYYRRWFAYWGQGTLVTVSS

SEQ ID NO: 97 - protein, 121 aa, Artificial Sequence
  Synthetic construct
QVQLQQSGPGLVKPSQTLSLTCAISGDSSNSAAWNWIRQSPSRGLEWLGRTYYSKWYNDYAVSVKSRITINPDTSKNQFSLQLNSVTPEDTAVYYCARYYDGYYRRWFAYWGQGTLVTVSS

SEQ ID NO: 98 - protein, 121 aa, Artificial Sequence
  Synthetic construct
EVQLQQSGPGLGRPGSSVKISCKASGYTFTGYILSWVRQSPSRGLEWIGWVDPEYGSTDSAEKFKKRATLNADISKNQAYLQLNSVTPEDTATYYCTRYYDGYYRRWFAYWGQGTTVTVSS

SEQ ID NO: 99 - protein, 121 aa, Artificial Sequence
  Synthetic construct
QVQLVQSGSELKKPGASVKVSCKASGYTFTSYAMNWVRQAPGQGLEWMGWINTNTGNPTYAQGFTGRFVFSLDTSVSTAYLQICSLKAEDTAVYYCARYYDGYYRRWFAYWGQGTLVTVSS

SEQ ID NO: 100 - protein, 121 aa, Artificial Sequence
  Synthetic construct
EVQLVQSGSELGRPGSSVKISCKASGYTFTGYILSWVRQAPGQGLEWIGWVDPEYGSTDSAEKFKKRATLSADISVNTAYLQLCSLKAEDTATYYCTRYYDGYYRRWFAYWGQGTLVTVSS

SEQ ID NO: 101 - protein, 17 aa, Artificial Sequence
  Synthetic construct
AEYFQHWGQGTLVTVSS

SEQ ID NO: 102 - protein, 17 aa, Artificial Sequence
  Synthetic construct
YWYFDLWGRGTLVTVSS

SEQ ID NO: 103 - protein, 15 aa, Artificial Sequence
  Synthetic construct
AFDVWGQGTMVTVSS

SEQ ID NO: 104 - protein, 15 aa, Artificial Sequence
  Synthetic construct
YFDYWGQGTLVTVSS

SEQ ID NO: 105 - protein, 16 aa, Artificial Sequence
  Synthetic construct
NWFDSWGQGTLVTVSS

SEQ ID NO: 106 - protein, 17 aa, Artificial Sequence
  Synthetic construct
YYGMDVWGQGTTVTVSS

SEQ ID NO: 107 - protein, 107 aa, Artificial Sequence
  Synthetic construct
VIWMTQSPSLLSASTGDRVTISCRMSQGISSYLAWYQQKPGKAPELLIYAASTLQSGVPSRFSGSGSGTDFTLTISCLQSEDFATYYCQQYYSFPITFGQGTKVEIK

SEQ ID NO: 108 - protein, 107 aa, Artificial Sequence
  Synthetic construct
VIWMTQSPSLLSASTGDRVTISCLASEGISNNLAWHQQKPGKAPELLIYGAHSLHDGVPSRFSGSGSGTDYTLTISCLQSEDFAVYYCQQGYKYPITFGQGTKVEIK

SEQ ID NO: 109 - protein, 107 aa, Artificial Sequence
  Synthetic construct
DVVMTQSPASLPVTLGQPASISCRSSQDGNTYLNWFQQRPGQSPRRLIYKVSNWDSGVPDRFSGSGSGTDFTLKISRVEAEDVGVYYCMQGTHWPITFGQGTKLEIK

SEQ ID NO: 110 - protein, 107 aa, Artificial Sequence
  Synthetic construct
DIVMTQSPLSLPVTLGPQVSISCLASEGISNNLAWHQQRPGQSPQRLIYGAHSLHDGVPDRFSGSGSGTDYTLKISRVEAEDVGVYYCQQGYKYPITFGQGTKLEIK

SEQ ID NO: 111 - protein, 107 aa, Artificial Sequence
  Synthetic construct
EIVLTQSPGTLSLSPGERVTLSCRASQVSSSYLAWYQQKPGQAPRLLIYGASSRATGIPDRFSGSGSGTDFTLTISRLEPEDFAVYYCQQYGSSPITFGPGTKVDIK

SEQ ID NO: 112 - protein, 107 aa, Artificial Sequence
  Synthetic construct
EIVMTQSPGTLSLSPGERATISCLASEGISNNLAWHQQKPGQAPQLLIYGAHSLHDGIPDRFSGSGSGTDYTLTISRLEPEDFAVYYCQQGYKYPITFGPGTKVDIK

SEQ ID NO: 113 - protein, 107 aa, Artificial Sequence
  Synthetic construct
DIVMTQSPDSLAVSLGERATINCKSSQNNKNYLAWYQQKPGQPPKLLIYWASTRESGVPDRFSGSGSGTDFTLTISSLQAEDVAVYYCQQYYSTPITFGGGTKVEIK

SEQ ID NO: 114 - protein, 107 aa, Artificial Sequence
  Synthetic construct
DIVMTQSPDSLAVSLGEKATINCLASEGISNNLAWHQQKPGQPPQLLIYGAHSLHDGVPDRFSGSGSGTDYTLTISSLQAEDVAVYYCQQGYKYPITFGGGTKVEIK

SEQ ID NO: 115 - protein, 107 aa, Artificial Sequence
  Synthetic construct
DVVMTQSPAFLSVTPGEKVTITCQASEGIGNYLYWYQQKPDQAPKLLIKYASQSISGVPSRFSGSGSGTDFTFTISSLEAEDAATYYCQQGNKHPITFGGGTKVEIK

SEQ ID NO: 116 - protein, 107 aa, Artificial Sequence
  Synthetic construct
DIVMTQSPAFLSVTPGEKVTITCLASEGISNNLAWHQQKPDQAPQLLIYGAHSLHDGVPSRFSGSGSGTDYTLTISSLEAEDAAVYYCQQGYKYPITFGGGTKVEIK

SEQ ID NO: 117 - protein, 12 aa, Artificial Sequence
  Synthetic construct
WTFGQGTKVEIK

SEQ ID NO: 118 - protein, 12 aa, Artificial Sequence
  Synthetic construct
YTFGQGTKLEIK

SEQ ID NO: 119 - protein, 12 aa, Artificial Sequence
  Synthetic construct
FTFGPGTKVDIK

SEQ ID NO: 120 - protein, 12 aa, Artificial Sequence
  Synthetic construct
LTFGGGTKVEIK

SEQ ID NO: 121 - protein, 12 aa, Artificial Sequence
  Synthetic construct
ITFGQGTRLEIK

SEQ ID NO: 122 - protein, 5 aa, Artificial Sequence
  Synthetic construct
GGGGS

SEQ ID NO: 123 - protein, 15 aa, Artificial Sequence
  Synthetic construct
GGGGSGGGGSGGGGS

SEQ ID NO: 124 - protein, 6 aa, Artificial Sequence
  Synthetic construct
HHHHHH

SEQ ID NO: 125 - protein, 8 aa, Artificial Sequence
  Synthetic construct
DYKDDDDK